European Patent Application EP 4 667 561 A1, published December 24, 2025. Title: 신규 락토코커스 락티스 아종 락티스 균주 및 이의 용도. Applicant: 주식회사 로렌츄컴퍼니. The sequence listing filed with the application follows.

SEQUENCE LISTING (33 sequences)

SEQ ID NO: 1 - RNA, 1459 nt, Lactococcus lactis
  source 1..1459: mol_type = rRNA
cgtgcctaatacatgcaagttgagcgctgaaggttggtacttgtaccgactggatgagcagcgaacgggtgagtaacgcgtggggaatctgcctttgagcgggggacaacatttggaaacgaatgctaataccgcataaaaactttaaacacaagttttaagtttgaaagatgcaattgcatcactcaaagatgatcccgcgttgtattagctagttggtgaggtaaaggctcaccaaggcgatgatacatagccgacctgagagggtgatcggccacattgggactgagacacggcccaaactcctacgggaggcagcagtagggaatcttcggcaatggacgaaagtctgaccgagcaacgccgcgtgagtgaagaaggttttcggatcgtaaaactctgttggtagagaagaacgttggtgagagtggaaagctcatcaagtgacggtaactacccagaaagggacggctaactacgtgccagcagccgcggtaatacgtaggtcccgagcgttgtccggatttattgggcgtaaagcgagcgcaggtggtttattaagtctggtgtaaaaggcagtggctcaaccattgtatgcattggaaactggtagacttgagtgcaggagaggagagtggaattccatgtgtagcggtgaaatgcgtagatatatggaggaacaccggtggcgaaagcggctctctggcctgtaactgacactgaggctcgaaagcgtggggagcaaacaggattagataccctggtagtccacgccgtaaacgatgagtgctagatgtagggagctataagttctctgtatcgcagctaacgcaataagcactccgcctggggagtacgaccgcaaggttgaaactcaaaggaattgacgggggcccgcacaagcggtggagcatgtggtttaattcgaagcaacgcgaagaaccttaccaggtcttgacatactcgtgctattcctagagataggaagttccttcgggacacgggatacaggtggtgcatggttgtcgtcagctcgtgtcgtgagatgttgggttaagtcccgcaacgagcgcaacccctattgttagttgccatcattaagttgggcactctaacgagactgccggtgataaaccggaggaaggtggggatgacgtcaaatcatcatgccccttatgacctgggctacacacgtgctacaatggatggtacaacgagtcgcgagacagtgatgtttagctaatctcttaaaaccattctcagttcggattgtaggctgcaactcgcctacatgaagtcggaatcgctagtaatcgcggatcagcacgccgcggtgaatacgttcccgggccttgtacacaccgcccgtcacaccacgggagttgggagtacccgaagtaggttgcctaaccgcaaggagggcgcttcctaaggtaagaccgatgactggggtgaagtc

SEQ ID NO: 2 - DNA, 20 bp, synthetic construct
  source 1..20: mol_type = other DNA
agagtttgatcctggctcag

SEQ ID NO: 3 - DNA, 17 bp, synthetic construct
  source 1..17: mol_type = other DNA
aaggaggtgatccagcc

SEQ ID NO: 4 - DNA, 27 bp, synthetic construct
  source 1..27: mol_type = other DNA
gttgtattagctagttggtgaggtaaa

SEQ ID NO: 5 - DNA, 20 bp, synthetic construct
  source 1..20: mol_type = other DNA
gttgagccactgccttttac

SEQ ID NO: 6 - DNA, 20 bp, synthetic construct
  source 1..20: mol_type = other DNA
cacaaggcagcaaatagacg

SEQ ID NO: 7 - DNA, 20 bp, synthetic construct
  source 1..20: mol_type = other DNA
gagttagcagtgaggcacca

SEQ ID NO: 8 - DNA, 22 bp, synthetic construct
  source 1..22: mol_type = other DNA
caggcgagaggagcacagatac

SEQ ID NO: 9 - DNA, 22 bp, synthetic construct
  source 1..22: mol_type = other DNA
tcctttcctacaagctcgtggg

SEQ ID NO: 10 - DNA, 24 bp, synthetic construct
  source 1..24: mol_type = other DNA
agagctgctcgagccaccaatgta

SEQ ID NO: 11 - DNA, 24 bp, synthetic construct
  source 1..24: mol_type = other DNA
caccaatctgatggccttcttcac

SEQ ID NO: 12 - DNA, 25 bp, synthetic construct
  source 1..25: mol_type = other DNA
gcgcttctattcctgctgctcacgg

SEQ ID NO: 13 - DNA, 24 bp, synthetic construct
  source 1..24: mol_type = other DNA
gtggcatcctggacccacttcttc

SEQ ID NO: 14 - DNA, 20 bp, synthetic construct
  source 1..20: mol_type = other DNA
tttgcctagaatccccacag

SEQ ID NO: 15 - DNA, 20 bp, synthetic construct
  source 1..20: mol_type = other DNA
taaggagcccagaaaacagc

SEQ ID NO: 16 - DNA, 24 bp, synthetic construct
  source 1..24: mol_type = other DNA
agagctgctcgagccaccaatgta

SEQ ID NO: 17 - DNA, 24 bp, synthetic construct
  source 1..24: mol_type = other DNA
caccaatctgatggccttcttcac

SEQ ID NO: 18 - DNA, 25 bp, synthetic construct
  source 1..25: mol_type = other DNA
gcgcttctattcctgctgctcacgg

SEQ ID NO: 19 - DNA, 24 bp, synthetic construct
  source 1..24: mol_type = other DNA
gtggcatcctggacccacttcttc

SEQ ID NO: 20 - DNA, 20 bp, synthetic construct
  source 1..20: mol_type = other DNA
gggtatggagaaggaggccc

SEQ ID NO: 21 - DNA, 20 bp, synthetic construct
  source 1..20: mol_type = other DNA
tccctgagccgaatcatcct

SEQ ID NO: 22 - DNA, 20 bp, synthetic construct
  source 1..20: mol_type = other DNA
agggcggtgaaatgaccatc

SEQ ID NO: 23 - DNA, 20 bp, synthetic construct
  source 1..20: mol_type = other DNA
cggcagcttcactgttgagg

SEQ ID NO: 24 - DNA, 20 bp, synthetic construct
  source 1..20: mol_type = other DNA
ctcagtggagttttaccggc

SEQ ID NO: 25 - DNA, 20 bp, synthetic construct
  source 1..20: mol_type = other DNA
aggtagacagcaccaccctg

SEQ ID NO: 26 - DNA, 17 bp, synthetic construct
  source 1..17: mol_type = other DNA
gagggttgccctccaga

SEQ ID NO: 27 - DNA, 20 bp, synthetic construct
  source 1..20: mol_type = other DNA
gcttgagcttctctgctgtt

SEQ ID NO: 28 - DNA, 23 bp, synthetic construct
  source 1..23: mol_type = other DNA
atcagtattgagcaccagccatt

SEQ ID NO: 29 - DNA, 23 bp, synthetic construct
  source 1..23: mol_type = other DNA
agagtgttgcctcgcaggtaaag

SEQ ID NO: 30 - DNA, 21 bp, synthetic construct
  source 1..21: mol_type = other DNA
cctgtcctgcgtgttgaaaga

SEQ ID NO: 31 - DNA, 20 bp, synthetic construct
  source 1..20: mol_type = other DNA
gggaactgggcagactcaaa

SEQ ID NO: 32 - DNA, 24 bp, synthetic construct
  source 1..24: mol_type = other DNA
agagctgctcgagccaccaatgta

SEQ ID NO: 33 - DNA, 24 bp, synthetic construct
  source 1..24: mol_type = other DNA
caccaatctgatggccttcttcac